European Patent Application EP 4 292 609 A1, published December 20, 2023. Title: Compositions comprising antibodies that bind gamma-delta T cell receptors. Applicant: LAVA Therapeutics. The sequence listing filed with the application follows.

SEQUENCE LISTING (18 sequences)

SEQ ID NO: 1 - protein, 5 aa, Artificial Sequence
  antibody sequence
  MISC_FEATURE (5)..(5): X is S or G
NYAMX

SEQ ID NO: 2 - protein, 17 aa, Artificial Sequence
  antibody sequence
AISWSGGSTSYADSVKG

SEQ ID NO: 3 - protein, 21 aa, Artificial Sequence
  antibody sequence
  MISC_FEATURE (7)..(7): X is F or S
QFSGADXGFGRLGIRGYEYDY

SEQ ID NO: 4 - protein, 130 aa, Artificial Sequence
  antibody sequence
  MISC_FEATURE (35)..(35): X is S or G
  MISC_FEATURE (105)..(105): X is F or S
EVQLLESGGGSVQPGGSLRLSCAASGRPFSNYAMXWFRQAPGKEREFVSAISWSGGSTSYADSVKGRFTISRDNSKNTLYLQMNSLRAEDTAVYYCAAQFSGADXGFGRLGIRGYEYDYWGQGTQVTVSS

SEQ ID NO: 5 - protein, 5 aa, Artificial Sequence
  antibody sequence
SYGMG

SEQ ID NO: 6 - protein, 17 aa, Artificial Sequence
  antibody sequence
GISWRGDSTGYADSVKG

SEQ ID NO: 7 - protein, 15 aa, Artificial Sequence
  antibody sequence
AAGSAWYGTLYEYDY

SEQ ID NO: 8 - protein, 124 aa, Artificial Sequence
  antibody sequence
EVQLVESGGGSVQPGGSLRLSCAASGRTSRSYGMGWFRQAPGKEREFVSGISWRGDSTGYADSVKGRFTISRDNAKNTVDLQMNSLRAEDTAVYYCAAAAGSAWYGTLYEYDYWGQGTLVTVSS

SEQ ID NO: 9 - protein, 5 aa, Artificial Sequence
  linker sequence
GGGGS

SEQ ID NO: 10 - protein, 14 aa, Artificial Sequence
  antibody sequence
AAASDKTHTCPPCP

SEQ ID NO: 11 - protein, 231 aa, Artificial Sequence
  antibody sequence
  VARIANT (231)..(231): X is K or absent
AAASDKTHTCPPCPAPEFEGGPSVFLFPPKPKDTLMISRTPEVTCVVVDVSHEDPEVKFNWYVDGVEVHNAKTKPREEQYNSTYRVVSVLTVLHQDWLNGKEYKCKVSNKALPAPIEKTISKAKGQPREPQVYTLPPSRDELTKNQVSLWCLVKGFYPSDIAVEWESNGQPENNYKTTPPVLDSDGSFFLYSKLTVDKSRWQQGNVFSCSVMHEALHNHYTQKSLSLSPGX

SEQ ID NO: 12 - protein, 231 aa, Artificial Sequence
  antibody sequence
  VARIANT (231)..(231): X is K or absent
AAASDKTHTCPPCPAPEFEGGPSVFLFPPKPKDTLMISRTPEVTCVVVDVSHEDPEVKFNWYVDGVEVHNAKTKPREEQYNSTYRVVSVLTVLHQDWLNGKEYKCKVSNKALPAPIEKTISKAKGQPREPQVYTLPPSRDELTKNQVSLSCAVKGFYPSDIAVEWESNGQPENNYKTTPPVLDSDGSFFLVSKLTVDKSRWQQGNVFSCSVMHEALHNHYTQKSLSLSPGX

SEQ ID NO: 13 - protein, 130 aa, Artificial Sequence
  antibody sequence
EVQLVESGGGLVQAGGSLRLSCAASGRPFSNYAMGWFRQAPGKEREFVAAISWSGGSTSYADSVKGRFTISRDNAKNTVYLQMNSPKPEDTAIYYCAAQFSGADYGFGRLGIRGYEYDYWGQGTQVTVSS

SEQ ID NO: 14 - protein, 130 aa, Artificial Sequence
  antibody sequence
EVQLLESGGGSVQPGGSLRLSCAASGRPFSNYAMSWFRQAPGKEREFVSAISWSGGSTSYADSVKGRFTISRDNSKNTLYLQMNSLRAEDTAVYYCAAQFSGADYGFGRLGIRGYEYDYWGQGTQVTVSS

SEQ ID NO: 15 - protein, 21 aa, Artificial Sequence
  antibody sequence
QFSGADYGFGRLGIRGYEYDY

SEQ ID NO: 16 - protein, 355 aa, artificial sequence
  antibody sequence
  VARIANT (355)..(355): X is K or absent
EVQLVESGGGSVQPGGSLRLSCAASGRTSRSYGMGWFRQAPGKEREFVSGISWRGDSTGYADSVKGRFTISRDNAKNTVDLQMNSLRAEDTAVYYCAAAAGSAWYGTLYEYDYWGQGTLVTVSSAAASDKTHTCPPCPAPEFEGGPSVFLFPPKPKDTLMISRTPEVTCVVVDVSHEDPEVKFNWYVDGVEVHNAKTKPREEQYNSTYRVVSVLTVLHQDWLNGKEYKCKVSNKALPAPIEKTISKAKGQPREPQVYTLPPSRDELTKNQVSLSCAVKGFYPSDIAVEWESNGQPENNYKTTPPVLDSDGSFFLVSKLTVDKSRWQQGNVFSCSVMHEALHNHYTQKSLSLSPGX

SEQ ID NO: 17 - protein, 361 aa, artificial sequence
  antibody sequence
  VARIANT (361)..(361): X is K or absent
EVQLLESGGGSVQPGGSLRLSCAASGRPFSNYAMSWFRQAPGKEREFVSAISWSGGSTSYADSVKGRFTISRDNSKNTLYLQMNSLRAEDTAVYYCAAQFSGADFGFGRLGIRGYEYDYWGQGTQVTVSSAAASDKTHTCPPCPAPEFEGGPSVFLFPPKPKDTLMISRTPEVTCVVVDVSHEDPEVKFNWYVDGVEVHNAKTKPREEQYNSTYRVVSVLTVLHQDWLNGKEYKCKVSNKALPAPIEKTISKAKGQPREPQVYTLPPSRDELTKNQVSLWCLVKGFYPSDIAVEWESNGQPENNYKTTPPVLDSDGSFFLYSKLTVDKSRWQQGNVFSCSVMHEALHNHYTQKSLSLSPGX

SEQ ID NO: 18 - protein, 361 aa, artificial sequence
  antibody sequence
  VARIANT (361)..(361): X is K or absent
EVQLLESGGGSVQPGGSLRLSCAASGRPFSNYAMSWFRQAPGKEREFVSAISWSGGSTSYADSVKGRFTISRDNSKNTLYLQMNSLRAEDTAVYYCAAQFSGADSGFGRLGIRGYEYDYWGQGTQVTVSSAAASDKTHTCPPCPAPEFEGGPSVFLFPPKPKDTLMISRTPEVTCVVVDVSHEDPEVKFNWYVDGVEVHNAKTKPREEQYNSTYRVVSVLTVLHQDWLNGKEYKCKVSNKALPAPIEKTISKAKGQPREPQVYTLPPSRDELTKNQVSLWCLVKGFYPSDIAVEWESNGQPENNYKTTPPVLDSDGSFFLYSKLTVDKSRWQQGNVFSCSVMHEALHNHYTQKSLSLSPGX